European Patent Application EP 4 484 565 A1, published January 1, 2025. Title: 一种酶法合成布瓦西坦手性中间体的方法. Applicant: 浙江工业大学. The sequence listing filed with the application follows.

SEQUENCE LISTING (6 sequences)

SEQ ID NO: 1 - DNA, 1020 bp, Paraburkholderia graminis
  source 1..1020: mol_type = genomic DNA
atgggtaaagttgtcaaagccgctgctgttcaattttctccagttctgtacagccgcgaagcaaccgtagcaaaagtcgtacagaagatccacgaactgggtctgaaaggcgtgcaattcgctaccttcccggaaaccgttgtcccgtactacccgtatttcgctgcagttcagactggtatcgagctgctgagcggttccgaacacctgcgtctgctggagcaggcggttactgttcctagcgcggctacggatgcaatcggtaaagctgctcgtgaagcaggtatggttgtatctatcggcgtgaacgagcgcgacggtggcacgctgtacaacacccaactgctgtttgatgccgatggcacgctgattcagcgtcgccgtaaaatcaccccaactcacttcgaacgtatgatttggggtcagggtgatggttctggtctgcgtgcggttgattccgccgtgggccgcattggtcagctggcgtgtttcgaacataacaacccactggcccgttacgcgatgatcgctgatggcgaacaaatccattctgcgatgtatccgggcagcgcttttggcgaaggttttgcgcagcgtatggaaatcaacattcgtcagcacgcactggaatccggcgcgttcgtagtcaacgcaaccgcatggctggatgcggatcagcaggcacaaattatgaaagacaccggctgcggcattggtccaattagcggtggttgtttcaccaccattgtttccccggacggtatgctgatggctgaaccgctgcgctctggtgagggcgaggtcatcgttgacctggactttgcacagatcgatcgtcgtaaaatgctgatggacgctgccggtcattacaaccgtccggaactgctgtctctgatgatcgatcgtacccctaccgcgcatgtacatgaacgtgcgccgcactccctgccggtaagcgacaaagcggacgacgacgtgcgcacccaagcggctgcagtcgcgggttcccgcctcgagatt

SEQ ID NO: 2 - protein, 340 aa, Paraburkholderia graminis
MGKVVKAAAVQFSPVLYSREATVAKVVQKIHELGLKGVQFATFPETVVPYYPYFAAVQTGIELLSGSEHLRLLEQAVTVPSAATDAIGKAAREAGMVVSIGVNERDGGTLYNTQLLFDADGTLIQRRRKITPTHFERMIWGQGDGSGLRAVDSAVGRIGQLACFEHNNPLARYAMIADGEQIHSAMYPGSAFGEGFAQRMEINIRQHALESGAFVVNATAWLDADQQAQIMKDTGCGIGPISGGCFTTIVSPDGMLMAEPLRSGEGEVIVDLDFAQIDRRKMLMDAAGHYNRPELLSLMIDRTPTAHVHERAPHSLPVSDKADDDVRTQAAAVAGSRLEI

SEQ ID NO: 3 - DNA, 1020 bp, Paraburkholderia graminis
  source 1..1020: mol_type = genomic DNA
atgggtaaagttgtcaaagccgctgctgttcaattttctccagttctgtacagccgcgaagcaaccgtagcaaaagtcgtacagaagatccacgaactgggtctgaaaggcgtgcaattcgctaccttcccggaaaccgttgtcccgtactacccgtatttcgctgcagttcagactggtatcgagctgctgagcggttccgaacacctgcgtctgctggagcaggcggttactgttcctagcgcggctacggatgcaatcggtaaagctgctcgtgaagcaggtatggttgtatctatcggcgtgaacgagcgcgacggtggcacgctgtacaacacccaactgctgtttgatgccgatggcacgctgattcagcgtcgccgtaaaatcaccccaactcacttcgaacgtatgattggcggtcagggtgatggttctggtctgcgtgcggttgattccgccgtgggccgcattggtcagctggcgtgtttcgaacataacaacccactggcccgttacgcgatgatcgctgatggcgaacaaatccattctgcgatgtatccgggcagcgcttttggcgaaggttttgcgcagcgtatggaaatcaacattcgtcagcacgcactggaatccggcgcgttcgtagtcaacgcaaccgcatggctggatgcggatcagcaggcacaaattatgaaagacaccggctgcggcattggtccaattagcggtggttgtttcaccaccattgtttccccggacggtatgctgatggctgaaccgctgcgctctggtgagggcgaggtcatcgttgacctggactttgcacagatcgatcgtcgtaaaatgctgatggacgctgccggtcattacaaccgtccggaactgctgtctctgatgatcgatcgtacccctaccgcgcatgtacatgaacgtgcgccgcactccctgccggtaagcgacaaagcggacgacgacgtgcgcacccaagcggctgcagtcgcgggttcccgcctcgagatt

SEQ ID NO: 4 - protein, 340 aa, Paraburkholderia graminis
MGKVVKAAAVQFSPVLYSREATVAKVVQKIHELGLKGVQFATFPETVVPYYPYFAAVQTGIELLSGSEHLRLLEQAVTVPSAATDAIGKAAREAGMVVSIGVNERDGGTLYNTQLLFDADGTLIQRRRKITPTHFERMIGGQGDGSGLRAVDSAVGRIGQLACFEHNNPLARYAMIADGEQIHSAMYPGSAFGEGFAQRMEINIRQHALESGAFVVNATAWLDADQQAQIMKDTGCGIGPISGGCFTTIVSPDGMLMAEPLRSGEGEVIVDLDFAQIDRRKMLMDAAGHYNRPELLSLMIDRTPTAHVHERAPHSLPVSDKADDDVRTQAAAVAGSRLEI

SEQ ID NO: 5 - DNA, 1020 bp, Paraburkholderia graminis
  source 1..1020: mol_type = genomic DNA
atgggtaaagttgtcaaagccgctgctgttcaattttctccagttctgtacagccgcgaagcaaccgtagcaaaagtcgtacagaagatccacgaactgggtctgaaaggcgtgcaattcgctaccttcccggaaaccgttgtcccgtactacccgtatttcgctgcagttcagactggtatcgagctgctgagcggttccgaacacctgcgtctgctggagcaggcggttactgttcctagcgcggctacggatgcaatcggtaaagctgctcgtgaagcaggtatggttgtatctatcggcgtgaacgagcgcgacggtggcacgctgtacaacacccaactgctgtttgatgccgatggcacgctgattcagcgtcgccgtaaaatcaccccaactcacttcgaacgtatgattggcggtcagggtgatggttctggtctgcgtgcggttgattccgccgtgggccgcattggtcagctggcgtgtttcgaacataacaacccactggcccgttacgcgaccatcgctgatggcgaacaaatccattctgcgatgtatccgggcagcgcttttggcgaaggttttgcgcagcgtatggaaatcaacattcgtcagcacgcactggaatccggcgcgttcgtagtcaacgcaaccgcatggctggatgcggatcagcaggcacaaattatgaaagacaccggctgcggcattggtccaattagcggtggttgtttcaccaccattgtttccccggacggtatgctgatggctgaaccgctgcgctctggtgagggcgaggtcatcgttgacctggactttgcacagatcgatcgtcgtaaaatgctgatggacgctgccggtcattacaaccgtccggaactgctgtctctgatgatcgatcgtacccctaccgcgcatgtacatgaacgtgcgccgcactccctgccggtaagcgacaaagcggacgacgacgtgcgcacccaagcggctgcagtcgcgggttcccgcctcgagatt

SEQ ID NO: 6 - protein, 340 aa, Paraburkholderia graminis
MGKVVKAAAVQFSPVLYSREATVAKVVQKIHELGLKGVQFATFPETVVPYYPYFAAVQTGIELLSGSEHLRLLEQAVTVPSAATDAIGKAAREAGMVVSIGVNERDGGTLYNTQLLFDADGTLIQRRRKITPTHFERMIGGQGDGSGLRAVDSAVGRIGQLACFEHNNPLARYATIADGEQIHSAMYPGSAFGEGFAQRMEINIRQHALESGAFVVNATAWLDADQQAQIMKDTGCGIGPISGGCFTTIVSPDGMLMAEPLRSGEGEVIVDLDFAQIDRRKMLMDAAGHYNRPELLSLMIDRTPTAHVHERAPHSLPVSDKADDDVRTQAAAVAGSRLEI